European Patent Application EP 4 674 946 A1, published January 7, 2026. Title: 新規遺伝子組換え用マーカー及びその利用. Applicant: 花王株式会社. The sequence listing filed with the application follows.

SEQUENCE LISTING (51 sequences)

SEQ ID NO: 1 - DNA, 624 bp, Starmerella bombicola
  source 1..624: mol_type = genomic DNA
atgtcgatagttgtgctgatttcgggtagcggaacaaatttgcaggctttaattgacgcgaagcttccgatttcccacgtcatttcaagttctgctgatgcctatggtcttgaaagagccagaagagccaacatttcaaccacaacgcataccctcaaaacctactatgggacaattcctgcttctgcaaaggacgaacggagagcagcgagagacagattcaacaaagagcttgcacaaataattatcgatttgaagccaacgctggtagtatgtgccggatggatgctgatcctttctccgatatttctcactcctctcgaacaacaaaacatagacatcatcaaccttcatcctgcgcttcctggtgcgtttcctggaatacatgctatccagagagcttgggaagctgggcagagaggagaaattaccaagggtggacttatgattcactatgtaattgccgctgttgacgaaggcaagccaatcctggttagagaaattgagctgaagaaggacgaaacggtagaacagtatgaggagagggtgcatgctgttgagcacgaggccattgtggaaggcacgaaaaaggcgcttgcatcacgcattcacaagggcatctag

SEQ ID NO: 2 - protein, 207 aa, Starmerella bombicola
MSIVVLISGSGTNLQALIDAKLPISHVISSSADAYGLERARRANISTTTHTLKTYYGTIPASAKDERRAARDRFNKELAQIIIDLKPTLVVCAGWMLILSPIFLTPLEQQNIDIINLHPALPGAFPGIHAIQRAWEAGQRGEITKGGLMIHYVIAAVDEGKPILVREIELKKDETVEQYEERVHAVEHEAIVEGTKKALASRIHKGI

SEQ ID NO: 3 - DNA, 24 bp, synthetic construct
  source 1..24: mol_type = other DNA
atgtcgatagttgtgctgatttcg

SEQ ID NO: 4 - DNA, 23 bp, synthetic construct
  source 1..23: mol_type = other DNA
ctagatgcccttgtgaatgcgtg

SEQ ID NO: 5 - DNA, 1128 bp, Starmerella bombicola
  source 1..1128: mol_type = genomic DNA
atgcaggacgatcagtacgctttggtcgttgataatggctctggtatgtgcaaggccggattcggcggtgaggaggcccctgccgccgtttttccatccgtcgtcggccgtcctcgccaccccggcatgatggttggcatgaaccagaaggacgcctacgtcggcgacgatgcgcagagcaagcgaggtattcttaacttgcgctacccgatcgagcacggtatcgtcaccaactgggacgatatggagaagatctggcaccacaccttctacaacgagctgcgccgtcttcccgaggagcaccagatcctcatgaccgaggccccgatgaacccgaagtctaaccgtaagaagatgacccagatcattttcgagaccttcaacgccccggccttctacgtggccatccaggcggttctttcgctgtacgccactggccgagtcaccggtattgttctcgattctggcgatggtgtcacccacgtcgtgcccatctactcgggctactcgatgaaccacgccatcaagcgtattgacctcgccggccgtgatttgaccgagtacctcatgaagctgctgaccgagcgtggcttcgccttcaccaccactgctgagcgtgaaatcgtgcgcgagatcaaggagaagctctgttacgtcgctcttgatttcgagcaggagatgcagaccgcagctcagtcgagctcgctggagaagaactacgagcttcccgacggccacgtcattaccatcggtaatgagcgcttccgatgccccgaggctctcttccacccggatgccctgggtctcgagtctgctggtattcacgagactactttccagagcatcatgaagtgcgacatcgacgtgcgtaaggagctctacggtaacatcgtcatctccggtggcaccaccatgtacccaggcatcgccgagcgtcttcagaaggagatcaccgctatggctccatcttcgatgaaggtcaagctcatcgccctgcccgagcgcaagtggatggtctggatgggtggctccattctctctgcccttggaactttccagcagatgtggatcaccaagcaggagtacgacgagaccggtccggaaatcgtccaccgccgctgtccctaa

SEQ ID NO: 6 - DNA, 24 bp, synthetic construct
  source 1..24: mol_type = other DNA
atgcaggacgatcagtacgctttg

SEQ ID NO: 7 - DNA, 21 bp, synthetic construct
  source 1..21: mol_type = other DNA
ttagggacagcggcggtggac

SEQ ID NO: 8 - DNA, 44 bp, synthetic construct
  source 1..44: mol_type = other DNA
cctcttaccaattgaactatggaaattaatgaagaattgggctg

SEQ ID NO: 9 - DNA, 46 bp, synthetic construct
  source 1..46: mol_type = other DNA
tcggacaacaattcatctgcagacatagccgaaattctactgtgag

SEQ ID NO: 10 - DNA, 47 bp, synthetic construct
  source 1..47: mol_type = other DNA
gccaagcttgcatgctccaatttctaaggcgcaagcgacgcttctag

SEQ ID NO: 11 - DNA, 25 bp, synthetic construct
  source 1..25: mol_type = other DNA
tcaattggtaagagggaacgcgtag

SEQ ID NO: 12 - DNA, 24 bp, synthetic construct
  source 1..24: mol_type = other DNA
tgaattgttgtccgaatgctctgc

SEQ ID NO: 13 - DNA, 46 bp, synthetic construct
  source 1..46: mol_type = other DNA
agagtcgacctgcagcccaacgccttgacaagctttccaaatagag

SEQ ID NO: 14 - DNA, 25 bp, synthetic construct
  source 1..25: mol_type = other DNA
gcatgcaagcttggcactggccgtc

SEQ ID NO: 15 - DNA, 27 bp, synthetic construct
  source 1..27: mol_type = other DNA
ctgcaggtcgactctagaggatccccg

SEQ ID NO: 16 - DNA, 20 bp, synthetic construct
  source 1..20: mol_type = other DNA
ctcttcgctattacgccagc

SEQ ID NO: 17 - DNA, 20 bp, synthetic construct
  source 1..20: mol_type = other DNA
cactttatgcttccggctcg

SEQ ID NO: 18 - DNA, 24 bp, synthetic construct
  source 1..24: mol_type = other DNA
tccaatttctaaggcgcaagcgac

SEQ ID NO: 19 - DNA, 23 bp, synthetic construct
  source 1..23: mol_type = other DNA
cccaacgccttgacaagctttcc

SEQ ID NO: 20 - DNA, 22 bp, synthetic construct
  source 1..22: mol_type = other DNA
catgattgagtgacgtacgatg

SEQ ID NO: 21 - DNA, 20 bp, synthetic construct
  source 1..20: mol_type = other DNA
cacagttccatacaagccag

SEQ ID NO: 22 - DNA, 3618 bp, Starmerella bombicola
  source 1..3618: mol_type = genomic DNA
atgacagatttcggaacccgcatagagcacactttcacatccggattcgaagggctcaggcgtcagtcaggatcccaattcgaacacattcagcttcacgactcgccttctcccaatcccgcagtcgctgattttagcgctcattccacttgcatggaggattcggcagctgccggtggtgcaaatcccaaggttccaagcaccgaagaactccaaaaggccgcaggtgcacctggtgcagctggtagcgaaccaatccctgccaaatctctggtgattaagacgaaaaagcctaggccatacgcttgtcctacgtgcacacgtagttttgctcgtttggagcatctcaaacggcatgagcgttcccacaccaaggagaaaccgtttcagtgtccggtgtgtgagcgcagctttgctagacgagaccttcttctgcgtcacaagcaaaaactccatgcgtctttctctccaacagaagaaaagcatcaagtcaaggactcacagttcccgggccaagtacctctggaccagggtcctgtccagtcgatcaggcagaccaacactggatcccagcctctcagtcaacatggcctatcacccctaaatgcgagggcaatggctcctgccaacgccatatatgctacctcggcacggttgctggcaaataatcaaacctcgtcgccctctccttccgttggcatgaacatgcaaaaccaaatggcccagctcatgcagaactacgaaggtatggacctgctcactcctcttcgctccacctcaccttcggaagctcaaatgcaaaatatgaatgctatgggtggtttgaacaactcaaacggctacatacctgctacagattcgttcaagcaagtcttccctcagcagacttcgttccctctgatgaactcccgcggtgaaaacaatttcggtgagtggaggcagctcaacccactcgcacacgagctcgaaatgcttcatggtgttgctccctcattcagagcagtctcgaatcgcccctctagagccagctccttcagtgctgcttcagctaccacataccttcgtgagaaggacctaaacttgtacccaacttcgcagcagtttggccaggaggcctcagaggtcggatttgccactcctcaggcgtacgctgtcgatgatgagggctacgatttcgagccattggacctgaacttcgtgtccccagctcagttgagccagccgccgccgcgtaagcgtcgggtgagccttcatacatcttcggcaagtcctatgatgaatgcgttccaagaaggaactccggcgataaacctaaatattcagcctcaaggacaaagccaagggcacctcgattctcctcaaccaggacctgcaatgctggcattgcgggcccaagcacgtacacagagacagctgtaccagaaccaccactttggctcgggaagcgttgagtctccgtcgtcattgagtttcttcgaatccggcgacaccattggcagtctgtcaggagttagccaaagcccatcaccacagcagcaccttgcgaaccagccgcagcagcctccaagtcagcagcctccaagccagcagcctccaagccagcagcaacaaactccgcaaacacagagacagccagcgtccagcaggcaacagtcgttggacagcttgttctctggcttagatagttcgtttggagagttttgtgggtctccaggcatgacgccagggttcacccctgagatggcgtccggaatgacgcctgcttttactcccagcatgcacgccccgtatcagaccagcatgtcgcctcttcctgaggaagccggtgatatcaaagactttatggcacagcagaacgacgacttcgtaaactcattatttgacgccgaaggtaaatcgcccgagctgcgtaaaagcggatactgttctgatagttataccgatagcagtggtttgaatgggagccatagtggcagcgccaatggcagcataaacggaagccacaccgggaatcatagcgaaagtcacaatggaagtcaccacggaaaccccaatggaggttttcatggcggtgtaagcttcgggattaacgatctgggcaacaacactaatagctcaggcagcaatgaggtcagcggaatgcagaggttcatggactcttacttcaacagcttcgatacacatttgtcatttgttcacaaagcctcacaggtctcacatgcgctctctgaattctcatcgaccatcggctctccagccatctctcctccatcttcgtcctcgtctgttggcaccaccgccgacacaagtttgaatgccaagcttgctctctcacaagcactggctgcagttggagcgcaaactttaggagagcgtggtgaagctcaggcatattattgggcagcacgcgaccataacaactcaggaagtaccactttggaagggctgcaggcagacattttagttgcggtacttggtttgttcttcgacgaaccttctgagcatgcagcttctttagataaactcacgtcatcgattacagagacggagttgattatcgctccactaacgaagtcccagaactactcaacttacgatagtggccatggccttggaggcgcccaatctctcaaagtttctgaggagtggccggctaacgctgagaggctttgggaccaatttattgccaaccaatcacgcgtcaggacgctccacgcattgcatgcaatttgctgttgggtgcgcagaccatctcagcagctactaaacgttctagaatcctgtggatgtgctccatgcgatgatgacctatggagagcacccaccagcgacatttggttgcgggtagttgcatcgaaagaactggatgcgcatcaggtcgccgaaacaggaggcaatcctcctcagcagttcagaatggtcttaaataagctgcgaaatggagaggtgccccaggaagttgtatcacagtttacgttacagtcgttactgttagctttagagctttcgtgtgaccctgcagaatactctttgcagtcttctagggcagcattgagggcctgggaaacgctttgggctcgaagcccagatgcctctctcgatcccagtccagagagtgggccgatcatgagtgattgtgtcggaattgtgtcgttggttgcattttcatctctgaaaatgcgtggtgttcttgatgctctgtggcaacatgactttgctaaggtcagtcaagaggtgtccaaggctgtcaagggacagcagtatagcgcctcctcagtcgctaattatgctgtggatactctcgtatggtgtgagggtcatgtttcatcccattcaatcttcttctctacactcctcgctgtttcggagtgtgggctggtgcttgccgagtccctacggctcatcatctcgaaaaacacgccaactagcaacgcagaggagcagcttatccaacgaagcaggaaacttgtgagtacagtgctcaaagtatcgccctctgccgacctcgagatgcttcccaatcacgttctgagagctgctgtgtgcttgattagactgagcgactggcctcttgttggtgctctttctcgcatgctgcttggtcacctgtcgacttga

SEQ ID NO: 23 - protein, 1205 aa, Starmerella bombicola
MTDFGTRIEHTFTSGFEGLRRQSGSQFEHIQLHDSPSPNPAVADFSAHSTCMEDSAAAGGANPKVPSTEELQKAAGAPGAAGSEPIPAKSLVIKTKKPRPYACPTCTRSFARLEHLKRHERSHTKEKPFQCPVCERSFARRDLLLRHKQKLHASFSPTEEKHQVKDSQFPGQVPLDQGPVQSIRQTNTGSQPLSQHGLSPLNARAMAPANAIYATSARLLANNQTSSPSPSVGMNMQNQMAQLMQNYEGMDLLTPLRSTSPSEAQMQNMNAMGGLNNSNGYIPATDSFKQVFPQQTSFPLMNSRGENNFGEWRQLNPLAHELEMLHGVAPSFRAVSNRPSRASSFSAASATTYLREKDLNLYPTSQQFGQEASEVGFATPQAYAVDDEGYDFEPLDLNFVSPAQLSQPPPRKRRVSLHTSSASPMMNAFQEGTPAINLNIQPQGQSQGHLDSPQPGPAMLALRAQARTQRQLYQNHHFGSGSVESPSSLSFFESGDTIGSLSGVSQSPSPQQHLANQPQQPPSQQPPSQQPPSQQQQTPQTQRQPASSRQQSLDSLFSGLDSSFGEFCGSPGMTPGFTPEMASGMTPAFTPSMHAPYQTSMSPLPEEAGDIKDFMAQQNDDFVNSLFDAEGKSPELRKSGYCSDSYTDSSGLNGSHSGSANGSINGSHTGNHSESHNGSHHGNPNGGFHGGVSFGINDLGNNTNSSGSNEVSGMQRFMDSYFNSFDTHLSFVHKASQVSHALSEFSSTIGSPAISPPSSSSSVGTTADTSLNAKLALSQALAAVGAQTLGERGEAQAYYWAARDHNNSGSTTLEGLQADILVAVLGLFFDEPSEHAASLDKLTSSITETELIIAPLTKSQNYSTYDSGHGLGGAQSLKVSEEWPANAERLWDQFIANQSRVRTLHALHAICCWVRRPSQQLLNVLESCGCAPCDDDLWRAPTSDIWLRVVASKELDAHQVAETGGNPPQQFRMVLNKLRNGEVPQEVVSQFTLQSLLLALELSCDPAEYSLQSSRAALRAWETLWARSPDASLDPSPESGPIMSDCVGIVSLVAFSSLKMRGVLDALWQHDFAKVSQEVSKAVKGQQYSASSVANYAVDTLVWCEGHVSSHSIFFSTLLAVSECGLVLAESLRLIISKNTPTSNAEEQLIQRSRKLVSTVLKVSPSADLEMLPNHVLRAAVCLIRLSDWPLVGALSRMLLGHLST

SEQ ID NO: 24 - DNA, 44 bp, synthetic construct
  source 1..44: mol_type = other DNA
tccggaattgacacaactatggaaattaatgaagaattgggctg

SEQ ID NO: 25 - DNA, 46 bp, synthetic construct
  source 1..46: mol_type = other DNA
taaatctagatgatatctgcagacatagccgaaattctactgtgag

SEQ ID NO: 26 - DNA, 42 bp, synthetic construct
  source 1..42: mol_type = other DNA
gccaagcttgcatgcgaaggggctctccgaagtacatcactg

SEQ ID NO: 27 - DNA, 32 bp, synthetic construct
  source 1..32: mol_type = other DNA
tgtgtcaattccggaaaaacgacagaaaagtg

SEQ ID NO: 28 - DNA, 35 bp, synthetic construct
  source 1..35: mol_type = other DNA
tatcatctagatttatatcacaagtcactatttac

SEQ ID NO: 29 - DNA, 44 bp, synthetic construct
  source 1..44: mol_type = other DNA
agagtcgacctgcagctcaatgaactgagacagcagcttgtcac

SEQ ID NO: 30 - DNA, 27 bp, synthetic construct
  source 1..27: mol_type = other DNA
gaaggggctctccgaagtacatcactg

SEQ ID NO: 31 - DNA, 29 bp, synthetic construct
  source 1..29: mol_type = other DNA
ctcaatgaactgagacagcagcttgtcac

SEQ ID NO: 32 - DNA, 21 bp, synthetic construct
  source 1..21: mol_type = other DNA
ctaaggccagtacaagagatc

SEQ ID NO: 33 - DNA, 26 bp, synthetic construct
  source 1..26: mol_type = other DNA
ctaaagctcgaattaatagagacacg

SEQ ID NO: 34 - DNA, 1815 bp, Starmerella bombicola
  source 1..1815: mol_type = genomic DNA
atgacggaagaggaggtccaacaggtatttcttggttttgtgcattctcgcattggttccttgagaatgtttgccacaggaatcaccagccttgctcttttagttgcctacagagtgtccccggagttgcgcaagactctcggggatgctgacacgcaccctcatcttcttagtatcaaggcaaaaatcaatacaaaagaggttatttggcatctgcccaaattcgcaatcccccctcctctaagtccaaatcagcctgcagcgataaccacggatgttgtgattgttggttccggttgctcaagtatggtggcttcttatcttttgacaaagaagggtttcaatgtgatcattgtggaaaaaggctaccacatcaatgcaattaccagtcccgaacacgacttccaacgtgacatcgaggcgtttgagggtgaacacaatatgacatctgcggatgcctcaacaatagttgttgcgggcgccacggtcggaggcggtggtgcagttaactggagctgttccttacgtccaactgagcttgttagacgtgagtttgtccagaaaggagctccactctatggctcgaaagagtttgaccacgctttggctgaggtcgaacgggttatgcaagtaagcactaagttcggtcttgagggtggcagcgataacgaacattcattcacgaacgatttgatcttgaaggccagcgagaagctcaattatcgagccaaggtcgcaggtcaaaatactgggaagcacagagcaaactctggcttcgtcgagtttggcagcagacagggcgaggctgaaggcggggtcgctgagtggttccgcaacagtttcaacaacggtgctcggttgctgcagagaggccacgttgtcaacatcaggcaccataacggttacgcctctggtgtagaggtagttgtagacgggtcaaagaccattttgataaactgcaaacgagttgtgtgcgctgcagggtcacttcagactccagtgctgctgcagaggtcaggtttcaagaactctcatatcggcaagggcctgaaattgcacccggtcactgcagcttatggtgtcttccccgaacagatagtgaacaagcgacttgatcccattatgaccacggtttgcacagaagtcgacaatctcgacggtgaaggccacgggccaaagatcgaggcgctgcaccacaggcctcttctcacatccttccctctgccataccgcgatgccaaggactttcaaaccaaggtggagagctgggagcatctttgcacgcttctggtcatcactcgtgataagggagaaggcaaagtgagcttttatcccccgaatccctcaaagccttatatcgaatacacgccgagcaagtatgatcttggggctctgctgaaagggtccctgtctgctgcgaacatgctttacgtacaaggcgcgcaacgcatattcttgtcaagcacattcatccccgatttcgtatccaataagccggtatctgagcgatcaatttgggacgacgactatcagaaatggtaccaggaggccaagcgcaaggaattcattctatatgacactaaagttgggtctgctcatcaaatgggtacctgtcgcatgagcgtgaacgggcccaagcatggcgccgttgacggaaagggacacctttacgagtgccccaatgttcacgttattgatacttcggtgtttcccgctgcttcgggcgtcaatccgatgataacgtgcatggctactgcttacgtgcttgcaaacaatcttatcgcggatctcactaagcttcaaactaagctatga

SEQ ID NO: 35 - protein, 604 aa, Starmerella bombicola
MTEEEVQQVFLGFVHSRIGSLRMFATGITSLALLVAYRVSPELRKTLGDADTHPHLLSIKAKINTKEVIWHLPKFAIPPPLSPNQPAAITTDVVIVGSGCSSMVASYLLTKKGFNVIIVEKGYHINAITSPEHDFQRDIEAFEGEHNMTSADASTIVVAGATVGGGGAVNWSCSLRPTELVRREFVQKGAPLYGSKEFDHALAEVERVMQVSTKFGLEGGSDNEHSFTNDLILKASEKLNYRAKVAGQNTGKHRANSGFVEFGSRQGEAEGGVAEWFRNSFNNGARLLQRGHVVNIRHHNGYASGVEVVVDGSKTILINCKRVVCAAGSLQTPVLLQRSGFKNSHIGKGLKLHPVTAAYGVFPEQIVNKRLDPIMTTVCTEVDNLDGEGHGPKIEALHHRPLLTSFPLPYRDAKDFQTKVESWEHLCTLLVITRDKGEGKVSFYPPNPSKPYIEYTPSKYDLGALLKGSLSAANMLYVQGAQRIFLSSTFIPDFVSNKPVSERSIWDDDYQKWYQEAKRKEFILYDTKVGSAHQMGTCRMSVNGPKHGAVDGKGHLYECPNVHVIDTSVFPAASGVNPMITCMATAYVLANNLIADLTKLQTKL

SEQ ID NO: 36 - DNA, 1617 bp, Starmerella bombicola
  source 1..1617: mol_type = genomic DNA
atgttaatcaaagacattattctaactccaatgagtttatccgctgttgctggcttgttgccactgctcttcgtagctttcttagttctacacgagcctatctggctcctatggtaccgctatgcagcacgtaggcacaagtgtagtatgcctcgcttcattgagaaatcgttcccactgggaatacaaagaaccatggacatgatcaagacggccaagtcatacaccttactggaagttcaatacgacagagtcttcaataagttcaaagcacggacgtatcttcgacaagctccccttcaataccaaatcttcacaatcgagccagaaaacattaagacaatcctggcaaccaaattcaatgattttggtcttggagcacgtttccacacagtgggaaaagtgtttggccaagggatatttacactcagcggaaatggatggaaacagtctcgatcgatgttgagacctcagttcactaaagatcaggtttgcagaattgatcagatttccagtcatgctgcggagttaataaaggagatgaaccgtgcaatgaaagtggaccaatttattgatgttcaacattatttccacaaacttacgctggatacagcgactgaattcctatttggggagtcctgcgagagcttgaaccctgagaatcagtcatgtattgtagcccgtgatggttcggagattactgccgaacaattcgtggagtcctacaactttctactgaattacgctttcaaacggaccctatcaagcaaagtctactggttgttcaactctaaggaattccgagatcacaagaaacgtgctcagtcctatattgactactacgttgataaggctctttacgccacatctttcgctgctgagaactctattgcagagaaggatgctgctgcagagtctagtggcatctatgtgttctcgcttgagatggctaaagttacccgagacccagtgacgatacgtgatcaaattttcaacattctcattgctggtagagatacaacagctgctacgttgagcttcgctattcatttccttgccagaaatcctgacgtattcaacaaactacgtgaggaggtcctcgatcattttggaaccaaggaggagcaaaggcctttatcattcgaacttctgaagcaagcaccttatttgaagcaagttataaatgaagtcttgcgtcttgcgccggtattgccattgaacttccgtactgctgtgagagatacaactctacccataggtggtggtcccgagcagaaggatccgatcttcgttcctaagggcaccgcagtttactattcaatttacatggtccacagggacatcaagtattggggtcctgacgcccacgaattcaatcccaatcgatgggagaacttgaagctagataatgtgtgggcattcttgcccttcaatggcggtccccgaatttgtctcggccaacaattcgccctgacagagctttcgctaactctggtgagactcttacaggagtattccaagattgagatgggtcccgacttcccagagtcccctcgtttctcaacaacgcttacagctcaacacgctcctcccggtgtggttgtgcggttttcttaa

SEQ ID NO: 37 - protein, 538 aa, Starmerella bombicola
MLIKDIILTPMSLSAVAGLLPLLFVAFLVLHEPIWLLWYRYAARRHKCSMPRFIEKSFPLGIQRTMDMIKTAKSYTLLEVQYDRVFNKFKARTYLRQAPLQYQIFTIEPENIKTILATKFNDFGLGARFHTVGKVFGQGIFTLSGNGWKQSRSMLRPQFTKDQVCRIDQISSHAAELIKEMNRAMKVDQFIDVQHYFHKLTLDTATEFLFGESCESLNPENQSCIVARDGSEITAEQFVESYNFLLNYAFKRTLSSKVYWLFNSKEFRDHKKRAQSYIDYYVDKALYATSFAAENSIAEKDAAAESSGIYVFSLEMAKVTRDPVTIRDQIFNILIAGRDTTAATLSFAIHFLARNPDVFNKLREEVLDHFGTKEEQRPLSFELLKQAPYLKQVINEVLRLAPVLPLNFRTAVRDTTLPIGGGPEQKDPIFVPKGTAVYYSIYMVHRDIKYWGPDAHEFNPNRWENLKLDNVWAFLPFNGGPRICLGQQFALTELSLTLVRLLQEYSKIEMGPDFPESPRFSTTLTAQHAPPGVVVRFS

SEQ ID NO: 38 - DNA, 1572 bp, Starmerella bombicola
  source 1..1572: mol_type = genomic DNA
atgattctttatgctgtgctgggcgcattcgccgccttcttgctttacatggatgtactttaccctttcgtgatttaccctctgagagcgcgatggcacaaatgtggttacatccctagagatttgagctggccattggggattccactcaccctggtagttctctcgaagttgaggaaagatatgctgctgcaattcatggcagcgcaagaccttagtcgcccttacaagacatccttacgtcaatttctgggtaaatgggtaatcgccactagagatcctgagaacatcaaggctgttctatccaccaagttcaatgacttctcgctgaaagaaagagggaataggatgaggcatgtaatcggtgatggaatttttacccaagatggcgcaccatggaagcactcgcgagatatgctcaggcctcagttcaccaaggatcaaatcagccgagtggaattgttgagccaccacatcgacgttttgattcgtgaaatcaggaagtcgggaggtaacgtcgagttgcaacgtttattccacctcatgactatggacaccgccactcactttctattcggcgagtccgttggctcgttggaggtcagtggcgaaagcaagggcattgagatcaccgacccaaagactggagagattgtgaacaccgttgattttgttgagtcttatacttttgcaaacaagtttgctctcaagaagattatcctcaacgacttggagtttttagccgacttgacggagccctcgtataagtggcatctgcgccgtgtccacacagtcatggatcactacgttcagctggctttgaaggctactgagaagtatgatcctgatgatgatagcgagaagggagaatactactttagccatgagctggcgaaactcacgagagaccccttgtcgttgagagatcagcttttcaatattctcattgctggccgcgacactaccgcagcaactttgtcctatgccttccactatctaacgaagaatcccgctatctacgccaaggtccgcgaagatgtgctcacggtcttccctaatggagacgcatcattggcgacttacgaggacttgcgaaaggctaagtatctccaaatggtgatcaaggaggtattgcgtcttgcgcctgcggttcccttgaacacgcgtgccgcggttcgtgacacatatctgccacggggcggaggcccagccggaaacctgcccgtttttgttcccaagggcactgctgtcaactaccctacatatattttgcaccgcgatccagatatctatggtgccgacgcgtacgagttcaaccccgagagatggaggcctgagaataagcttccgaatagcccaatgtactcttggggatacattcccttcaatggtggccctcgcatctgcattggacagcagttcgccttgactgagatcgctttgacgatgatcaagctggttctggaatttgagaggctggagcctgccgacgactttgagcccaatcttcaagacaagtcctctttaactgtcatggtcggagggtcgggcgtccgagtgaaactgagttaa

SEQ ID NO: 39 - protein, 523 aa, Starmerella bombicola
MILYAVLGAFAAFLLYMDVLYPFVIYPLRARWHKCGYIPRDLSWPLGIPLTLVVLSKLRKDMLLQFMAAQDLSRPYKTSLRQFLGKWVIATRDPENIKAVLSTKFNDFSLKERGNRMRHVIGDGIFTQDGAPWKHSRDMLRPQFTKDQISRVELLSHHIDVLIREIRKSGGNVELQRLFHLMTMDTATHFLFGESVGSLEVSGESKGIEITDPKTGEIVNTVDFVESYTFANKFALKKIILNDLEFLADLTEPSYKWHLRRVHTVMDHYVQLALKATEKYDPDDDSEKGEYYFSHELAKLTRDPLSLRDQLFNILIAGRDTTAATLSYAFHYLTKNPAIYAKVREDVLTVFPNGDASLATYEDLRKAKYLQMVIKEVLRLAPAVPLNTRAAVRDTYLPRGGGPAGNLPVFVPKGTAVNYPTYILHRDPDIYGADAYEFNPERWRPENKLPNSPMYSWGYIPFNGGPRICIGQQFALTEIALTMIKLVLEFERLEPADDFEPNLQDKSSLTVMVGGSGVRVKLS

SEQ ID NO: 40 - DNA, 1671 bp, Starmerella bombicola
  source 1..1671: mol_type = genomic DNA
atgaggcccctgttgcgggaacaagacacatcacacccagagctattgttggcaagcaatactatttttaaccccctttccaagagtgtccaaactgttcaatacggcctcatgaacattaatttctctgacgtgctcgtgctaggaggcatcagcgtgagctttttgctcgcctaccaggcgatttacttttatttcatttactcgccacgagccaaaaagctcggttgcgctcttccaccggtcttcttctctttcccactcggaataccggaggtcatacgtcttgtgaacgcctggttcaacgatgatctccttgagtatttcaccttcaaattcgaggagttccagcgcaaaaccggattccaatcagtcgctgggcaactatggattgggactattgagcccgagaacatcaagactatgctcgctacttcatttaaagactactccctaggcttccgttacgaggccatgtacggccttctcggaaatggcattttcactctcagtggtgagggctggaagcacagccgcgctttgttgcgtccgcaatttagtcgtgagcaagtctctcaccttgaatcaatgcgcacacacatcaatatgttgatcaacaaccacttcaagggtggcaaagtcgtcgatgctcaggttttgttccacaatctaaccattgatactgctaccgaattcctattcggagagagcaccaacactcttgaccctgctcttgctcagcatggattccctggacctaagggtcttgtaaccggtgagcagtttgctgaggcttttacctctgctctcgaattgctttctgtgcgagttatggccggcgccgcatggttcctcgtttggacccccaaattctggcgctcatgcaaagtctgccacaacttcattgattacttcgttttcaaggctctggccactcctatggagaaggaccaggaagctgatcgctacgtctttattcgagaactcacaaaggagacctctgacccacgggtcatccgcgaccaggccctcaacatcctcttggctggtcgtgataccactgcggcacttctcagcttcaccacctactaccttggtgcctaccctgaggtctacgatgagcttcgcgaggctgttattgcggacttcggcaaggaagatgctgagccccctacgtttgagcagcttaagcagtgcaaggtgctacagaacgtcattcgggaagttttgcgattgcacccgaatgtgcccctcaacttccgcgaggccattaccgatactaagttccccacaggaggcggcccgaatggagaccagcccgttttcgttcccaagggacagaaagtgttttacgccacctacgtcatgcagcgaaatgagggtctctggggtcctgactccacaacattccgccctgaccgctggaacgagtcaagagaggccatcgcatccggatgggactacattcctttcaacggcggccctcgtatttgcctgggtcagcagttcgctctcacagaggcgagctacacgctcgtgcgtatctgccaagagttctccaggattgaggttctccaccctgatgttattacctccaggaacgtgatgaaacagcgcatgcgtttgaccaactcttccagcggcggcgtcatagcgaagttcattcgctag

SEQ ID NO: 41 - protein, 556 aa, Starmerella bombicola
MRPLLREQDTSHPELLLASNTIFNPLSKSVQTVQYGLMNINFSDVLVLGGISVSFLLAYQAIYFYFIYSPRAKKLGCALPPVFFSFPLGIPEVIRLVNAWFNDDLLEYFTFKFEEFQRKTGFQSVAGQLWIGTIEPENIKTMLATSFKDYSLGFRYEAMYGLLGNGIFTLSGEGWKHSRALLRPQFSREQVSHLESMRTHINMLINNHFKGGKVVDAQVLFHNLTIDTATEFLFGESTNTLDPALAQHGFPGPKGLVTGEQFAEAFTSALELLSVRVMAGAAWFLVWTPKFWRSCKVCHNFIDYFVFKALATPMEKDQEADRYVFIRELTKETSDPRVIRDQALNILLAGRDTTAALLSFTTYYLGAYPEVYDELREAVIADFGKEDAEPPTFEQLKQCKVLQNVIREVLRLHPNVPLNFREAITDTKFPTGGGPNGDQPVFVPKGQKVFYATYVMQRNEGLWGPDSTTFRPDRWNESREAIASGWDYIPFNGGPRICLGQQFALTEASYTLVRICQEFSRIEVLHPDVITSRNVMKQRMRLTNSSSGGVIAKFIR

SEQ ID NO: 42 - DNA, 1299 bp, Starmerella bombicola
  source 1..1299: mol_type = genomic DNA
atggccatcgagaaaccagtgatagttgcttgtgcctgcccactagcggggcacgtgggcccagtgctcagcctggtccgcggtctactcaatagaggatatgaggtgactttcgtaacagggaacgcattcaaggagaaagttattgaggcaggatgcactttcgtccctctccaaggacgagctgactaccatgaatacaatctccctgaaatcgctccaggattgctcacgattcctccaggccttgagcagaccggttactcaatgaatgagatttttgtgaaggcgattcctgagcagtacgatgcacttcaaactgctctaaaacaggttgaggctgaaaataaatcagctgtggtgattggcgagaccatgtttctaggggtgcatccgatatcactgggtgccccaggtctcaagccccaaggcgtaatcacgttaggaactattccgtgcatgctgaaagcagagaaggcgcctggagttcctagtcttgagccaatgattgatactttagtgcggcaacaagtatttcaaccaggaactgactctgagaaggagatcatgaagacgctcggggccacgaaggagcccgaatttctcctggagaatatatacagcagccctgacagatttttgcaactgtgccctccatctcttgaatttcacttgacttcgcctcctcctggcttctcgttcgctggtagtgcaccgcatgtaaagtctgctggattagcaactccacctcacctgccgtcttggtggcctgatgtgctgagtgcgaagcgtctgattgttgttacacaaggaacagcagccatcaactatgaagatctgctcattccagcattgcaggcctttgctgacgaagaagacactctcgtagttggtatattgggcgtcaaaggggcgtcacttcctgatagcgttaaagttcctgcaaacgctcgaattgttgattattttccttacgatgagctactaccgcatgcctctgttttcatatacaacggtggatacggaggtctgcagcacagtttgagccatggcgttcccgtcatcatcggaggaggaatgttggtagacaagccagctgttgcttcacgagctgtatgggctggtgttggttatgatcttcaaaccttgcaggcaacttctgagctagtctccacggccgttaaggaggtgttggctactccctcgtatcacgagaaagccatggcagtcaagaaagagcttgaaaaatacaagtctcttgatattctagagtcggcaattagtgaattagcttcttaa

SEQ ID NO: 43 - protein, 432 aa, Starmerella bombicola
MAIEKPVIVACACPLAGHVGPVLSLVRGLLNRGYEVTFVTGNAFKEKVIEAGCTFVPLQGRADYHEYNLPEIAPGLLTIPPGLEQTGYSMNEIFVKAIPEQYDALQTALKQVEAENKSAVVIGETMFLGVHPISLGAPGLKPQGVITLGTIPCMLKAEKAPGVPSLEPMIDTLVRQQVFQPGTDSEKEIMKTLGATKEPEFLLENIYSSPDRFLQLCPPSLEFHLTSPPPGFSFAGSAPHVKSAGLATPPHLPSWWPDVLSAKRLIVVTQGTAAINYEDLLIPALQAFADEEDTLVVGILGVKGASLPDSVKVPANARIVDYFPYDELLPHASVFIYNGGYGGLQHSLSHGVPVIIGGGMLVDKPAVASRAVWAGVGYDLQTLQATSELVSTAVKEVLATPSYHEKAMAVKKELEKYKSLDILESAISELAS

SEQ ID NO: 44 - DNA, 1392 bp, Starmerella bombicola
  source 1..1392: mol_type = genomic DNA
atgagcccttcatcacacaaacccctgattctcgcttgcggcttgcctctttcaggccatataatgcccgttttgagtctggtacacggccttacggacgacggatacgaagctactgttgtgacaggcagagcgtttgaacaaaaagttcgagatgtgggtgcagactttgttcctttagaagggaacgcagattttgatgaccacaccttagacgatctggtcccgggccgtaaagacatggccccaagcttcgatcgtacagttcaagatgtggagcacatgatggtagctactcttcctgagcagtttgccgctattcagagggctttcaaaaagctcagcgcaagcggccgccctgtcgttcttgtcagtgaagtgctgtttttcggtgcacaccctatcagcctcggtgctcctggtttcaaacccgctggctggatttgtttaggggttttgcctcttttgatccgcagtgatcataccttaggacttgacaacgacaggagccccgaagcacatgcaaagaaactcgctatgaaccacgctcttgagcaccaaattttcgttaaagccactgctaagcacaaggaaatctgccgagagttaggttgcactgaagatcccaaatttatctgggagcacagttacattgctgcagacaagttcctgcagctgtgcccgccttctcttgagttcagcagagaccatctgcctagcaacttcaaattcgccggctcaacgcccaagcaccgaactcaattcacccctccttcctggtggggggatgttctgagtgccaagcgagtcatcatggtcactcaaggaacttttgctgtcagttacaagcatcttattgtgcctactcttgaggccttgaaggacgagcctgacactttaacagtagccatattgggccgccgcggtgccaagctaccggatgatgttgtggttcctgagaatgctcgcgtgatcgactacttcaactacgatgctctacttcctcacgttgatgctcttgtctacaatggtggatatggcggacttcagcacagcttaagccactctgttccagttgttattgctggtgactctgaagacaagccaatggtggcatcgagagctgaggccgctggcgtggcaattgatttgaaaactggcttgcctacagtggagcaaatcaaagaagctgttgattcgataattggaaatccgaaattccacgaagcctcgaagaaggttcaaatggagttggaaagccacaactccttgaaaattcttgaggaaagcatcgaggaaatcgccagccatgactttggtcttttgaccaagagtgacgaggaaactgaagatatacctgtcaaagggccggccttagcggtgagttcttag

SEQ ID NO: 45 - protein, 463 aa, Starmerella bombicola
MSPSSHKPLILACGLPLSGHIMPVLSLVHGLTDDGYEATVVTGRAFEQKVRDVGADFVPLEGNADFDDHTLDDLVPGRKDMAPSFDRTVQDVEHMMVATLPEQFAAIQRAFKKLSASGRPVVLVSEVLFFGAHPISLGAPGFKPAGWICLGVLPLLIRSDHTLGLDNDRSPEAHAKKLAMNHALEHQIFVKATAKHKEICRELGCTEDPKFIWEHSYIAADKFLQLCPPSLEFSRDHLPSNFKFAGSTPKHRTQFTPPSWWGDVLSAKRVIMVTQGTFAVSYKHLIVPTLEALKDEPDTLTVAILGRRGAKLPDDVVVPENARVIDYFNYDALLPHVDALVYNGGYGGLQHSLSHSVPVVIAGDSEDKPMVASRAEAAGVAIDLKTGLPTVEQIKEAVDSIIGNPKFHEASKKVQMELESHNSLKILEESIEEIASHDFGLLTKSDEETEDIPVKGPALAVSS

SEQ ID NO: 46 - DNA, 780 bp, Starmerella bombicola
  source 1..780: mol_type = genomic DNA
atggttgtaaactcctcgaaggaccctcaaaacaaaggaatgactcctagaaaagaaattgaccaggaaatggtctcttgggccaaaaaaaacctcaaaaacacccctggcaatgaaaactatgagaagatggtctcaggagttccttacaatccatacgatccagatcttatgtttagagccctggctactagtgagaaagttagggagttcaataccattgcaagtgaaagtcgtacttttgagtcaaatcacgctgcttatatcaagaaggtcgagattctcaaagacacttttggtcaaacaaaggatattgtctggctgaccgctccattctcagttgattttggattcaacatcagcgtaggcgagcacttttacgccaacttcaacgtttgcttcttggactcggctccaataatctttggtgatgaggtgattgtagggcccaatacaacgttcgtgactgcgactcatcctattagccccgagaaacgtgcgaggagaattgtgtatgctcttcctatcaaggtggggaataatgtatggattggtgcgaatgtgactgtcctgccgggtgttacgattggagatggctcaacaattgcggctggtgctgtcgttcgagaagatgttcctcctcgtactgtggtgggaggagtccctgcgcgaatcctcaagcatattccagaggaggatcccgacgaggctgaaggagaggaactggaattccttcttccagttgaaatgaacgtcaataccgctaaccagaaggtctag

SEQ ID NO: 47 - protein, 259 aa, Starmerella bombicola
MVVNSSKDPQNKGMTPRKEIDQEMVSWAKKNLKNTPGNENYEKMVSGVPYNPYDPDLMFRALATSEKVREFNTIASESRTFESNHAAYIKKVEILKDTFGQTKDIVWLTAPFSVDFGFNISVGEHFYANFNVCFLDSAPIIFGDEVIVGPNTTFVTATHPISPEKRARRIVYALPIKVGNNVWIGANVTVLPGVTIGDGSTIAAGAVVREDVPPRTVVGGVPARILKHIPEEDPDEAEGEELEFLLPVEMNVNTANQKV

SEQ ID NO: 48 - DNA, 1233 bp, Starmerella bombicola
  source 1..1233: mol_type = genomic DNA
atgctggctctgtttttttcgcttgcgcctctactttctcaagctctccctttaggctatactgcggcccccgctgaatcattctatttttggccagagaacatatccagcctccaagctggcgagatttttagaaaacgggaactcttaactctcccagacatctttgactttggccctaatctggaaaaggtcgtacaagtggcttacaaaacccgtctcaccgatggcaatgactcgttttccatcgccagtatctttatccctaagaatccaagcccagaactcaaactttactcttatcagacgtttgaggatgccgtgcagcttgattgtgccccaagctatgctttagaagtgggtaacaagtccagcaactatcttcctgtcactagcaatttatctgccatcagtcgagaacttgagaaaggacgtcactgcattatccctgatcacgagggctatatttcaggattctttgcaggacggcaggagggatatgctggtttagacggaattcgcgctgctcgaaactatctcaatggcaccaacgagaccccaattggtatcttcggatacagtggaggtgcacaagcaacggcctggattgttgatttgcatgacgagtatgctcctgacttgaactttgttggaacagtttctggaggcactttggttgacgcttggggcacttttcagtatatcgactatccgaaggtgtatctaaagggcagcattcttatcatgtatacgggtcttttttcaggttatccagctcaatttgaggtgatttggccatatattgagcctgtaattcaagaaaacatgctactgctacgtttggcgccgaatgattgtaaccaaagcccgatacttcaaggttacaacaattcaatcatggccggtatacatgtggaccttcccgaattccctgcttctaagtacatattccagcacgagtccctccttgccaactacagcgtagtgccagtttccacaccgaagtttcctcgctacatgtaccatggtggatctgatgagttggccaaattgagccttgtcgagcagtatgttgatcaacaatggaataccggcgctaatctcaccttcgtggtgtatccgggtcttcttcatgacgagacggcttaccgtggctttgatgccgcgatggattggcttgatgcccagctcgatagtggataccttccacctgtaaactcaactcatacatga

SEQ ID NO: 49 - protein, 410 aa, Starmerella bombicola
MLALFFSLAPLLSQALPLGYTAAPAESFYFWPENISSLQAGEIFRKRELLTLPDIFDFGPNLEKVVQVAYKTRLTDGNDSFSIASIFIPKNPSPELKLYSYQTFEDAVQLDCAPSYALEVGNKSSNYLPVTSNLSAISRELEKGRHCIIPDHEGYISGFFAGRQEGYAGLDGIRAARNYLNGTNETPIGIFGYSGGAQATAWIVDLHDEYAPDLNFVGTVSGGTLVDAWGTFQYIDYPKVYLKGSILIMYTGLFSGYPAQFEVIWPYIEPVIQENMLLLRLAPNDCNQSPILQGYNNSIMAGIHVDLPEFPASKYIFQHESLLANYSVVPVSTPKFPRYMYHGGSDELAKLSLVEQYVDQQWNTGANLTFVVYPGLLHDETAYRGFDAAMDWLDAQLDSGYLPPVNSTHT

SEQ ID NO: 50 - DNA, 3900 bp, Starmerella bombicola
  source 1..3900: mol_type = genomic DNA
atggtggatgatatacaggtagagaagcgtgagaaactcatcgagactaaggacaagcttctcgaggagaagctctctgcgttagatccacatgaggccaatgtattgcgaagtcagcttgaaacaaagagagtcgccacaagctttttcaggttgttcagattttgcactccccttgacgttttcttggagatacttgcgcttttttttgcagcggtgcatggagccgcgcttccaatgttcacgttagtagtgggcgccatcttcaacacattcagagacttcacttcatatgacctcaagggcaatgagttccagcataaggtgaatcacctgtctctctattttgtctatattggcattggtatgctcggcagtgcgtttctcgagagcttcctgcttgtggacagaggcgaagtgttggcaggacgttaccgaaagcattatctgagtgctgttattcgccagaatatcgcgttttacgacaaactaggtggtggcgaggtcagcaccagaatcattaacgataccaactcaattcaggaagcgatcagcgacaagcttggaaacgtcgtacagggaatagcttccttcattgcggccaccgttataagttttgcttcgcaatggaaactggcttgcatcctcctgagtgctgtagggttcatggtaatcacaatgggaactggcgccaccttcatggccaaatatcagctcagatctgacgcgatatattcgcagtctggagctaccgttgcggaggaggctctcagtgctgtcaggactacagtagcatttggcgctcaacctcatctcgccgtcaagtatgaaaaggtacttgatcgtgttgtgaaggaatcgaagcggagcagttactcattgggggtcatgttagcgtgcatatgggctagtactttttgggtgtatgccttagctctgtggcagggttccagagaaatcgttagtgggagtgctgacgttggaaagataatagttgtaatcacagctatgttacttggaagcttccagcttgggaatatcgcgccaaacgtgaggtttcttgtcaagggtctcactgccgcgagcattctcaatgaggccattgatcgtgtcccagtcatcgatggccagtccatagataaaggaattgtcccccaaactaaggccgttggcagaattgagctcaaaaatgtcaagttccgatatcctagtcgcccagacgttttggtcctctccgattttagccttgaagttcctgctggatctactgtggcactggtaggtgcctcgggatcagggaagtctacaattgtaggtattcttgagaggttctatttacctctcgaaggaagcgttactctggatggccaggagattagcgacctgaacacaagatggctccgtcaacaaattggttatgttcagcaggaaccagtactcttttcagagtcaatatatgagaatatcagctatggtttgattggcactgacattgagttcgctgacgagcatgttaaggaagctaaaatcattcaagcttgtaaagatgccaatgcctgggatttcattcagactctctcagaaggcatccaaaccaatgttggagatcgaggatttcttctcagcggtggtcagaaacaacgcattgcaatagcaagagcaatcgtctcagaccctaaaattctgctgctcgatgaagcgacttctgctctggataccaaatctgaaggtatcgttcaagatgcgctcgacaaagcggccgaaggtcgtaccactatagtcgttgcacacagactctctacgatcaaggatgccaacaagatagttgtcatgtctaaaggtaacgtcatagagcagggtactcacaatgagctcatacagcgagaagggccttataaagctttggttgatgctcaaagagtaactaaagcaaagagcactaacgttgaggtcctcgatattgaagctctagacatttcgcctctggactcactgaacgaaaagttcaatcccaaggatgtgagcacattgagtgttcacagtgcaggtactcagaccactcaacctcctgaatatcaagaaaatgacatccctggtgtgcgcaaccccccacatagcacgttgatgaccaataccaaactggtttgggggctgaataggaaagaatggggttacattctcattggtagtttagcctccattattttgggctattgctatcctgcaatggcaataataactggccaaaccactggaagcatggttctacctcccagtgaatacggaaaaatgcggcatgtggtgaatatcatgggatggtggtattttttcgtaggctgcatttcattcatgacggcttttatcactatagctgctttatcacttgcatctgataagttggtcaaaaatatcagattagctttgttccgccaattgatgcgaatggatattgcattcttcgaccacaaaaacaacacgccgggtgcgctaacctcaattttggcgaaggaagctaaaatgatcgagggtttgagtggggccaccctcggtcaaattcaacagagtctggtgaccttgattggcggcatagttactggtatacctttcaattggagaattggactcgtggctacgtctgttgttcctgtcatgttggtgtgtggcttcgtcagagtctgggttcttacccaattatcggatcgtgcgagagaagtttacgaacgaagtggctccatggcatctgagtatacaagtgctgtccgcacagtccagtccttaactcgtgagttagacgtggtcgtaaaatacacaaagacagtagactctcagattttcagctccagaattgccattgcccgctcagcattgtactacgcactctcggaaggaatgacaccctgggtggtagccctcgttttttggtggggaagcactgtaatgagacgaggtgaagcttcggtcgcaggatatatgactgtcttcatggctattattacaggttctcaagccgctggccaaattttcagctatgctccaaacatgaactcagccaaagatgcagcgcgtaacatttacagaatcttgactgccactccttctatagatgtatggagtgaggaaggttacgttgctcccgaggagtcggtgagaggagatattgagttccgtcatgtgaatttccgatatcctactcgacctcaagtaccagttttacaagatctcaacttaacagtcaaaaagggccaatacatcgctctagttggagccagtggatgcggtaagtctactactattggactggtggaaagattttatgatccattagcaggtcaagtacttttcgatgggaaagatttacgcgaatataacctgaatgcattgagatcacacattgctttagtccagcaagaaccaatgctttattcaggcacgctacgtgagaatattctaatgggatggtctggccctgagtctgaagtaacgcaggagatgattgaggatgccgctcgcaaagcgaacattcacgaattcatcatgtcgttgcctgatggctacgaaacgctcagcggatctaggggatcgttgctatctggggggcaaaagcagcgaattgcaattgcaagggccctgatcagaaatccaaaggtactcctcctcgatgaggccacctcagctctggattccgaatctgagaaagtagttcaagcagcactcgacgcagcagcgaagggccgtactacaatcgccgttgcgcatagattatcaacaattcagaaagcagatgtcatatatgtgttctcaggagggcgcatcgtggagcagggcgaccatcagagcctccttgaactcaatggatggtacgctgaattggtgaacttgcaaggtctcggagagatttga

SEQ ID NO: 51 - protein, 1299 aa, Starmerella bombicola
MVDDIQVEKREKLIETKDKLLEEKLSALDPHEANVLRSQLETKRVATSFFRLFRFCTPLDVFLEILALFFAAVHGAALPMFTLVVGAIFNTFRDFTSYDLKGNEFQHKVNHLSLYFVYIGIGMLGSAFLESFLLVDRGEVLAGRYRKHYLSAVIRQNIAFYDKLGGGEVSTRIINDTNSIQEAISDKLGNVVQGIASFIAATVISFASQWKLACILLSAVGFMVITMGTGATFMAKYQLRSDAIYSQSGATVAEEALSAVRTTVAFGAQPHLAVKYEKVLDRVVKESKRSSYSLGVMLACIWASTFWVYALALWQGSREIVSGSADVGKIIVVITAMLLGSFQLGNIAPNVRFLVKGLTAASILNEAIDRVPVIDGQSIDKGIVPQTKAVGRIELKNVKFRYPSRPDVLVLSDFSLEVPAGSTVALVGASGSGKSTIVGILERFYLPLEGSVTLDGQEISDLNTRWLRQQIGYVQQEPVLFSESIYENISYGLIGTDIEFADEHVKEAKIIQACKDANAWDFIQTLSEGIQTNVGDRGFLLSGGQKQRIAIARAIVSDPKILLLDEATSALDTKSEGIVQDALDKAAEGRTTIVVAHRLSTIKDANKIVVMSKGNVIEQGTHNELIQREGPYKALVDAQRVTKAKSTNVEVLDIEALDISPLDSLNEKFNPKDVSTLSVHSAGTQTTQPPEYQENDIPGVRNPPHSTLMTNTKLVWGLNRKEWGYILIGSLASIILGYCYPAMAIITGQTTGSMVLPPSEYGKMRHVVNIMGWWYFFVGCISFMTAFITIAALSLASDKLVKNIRLALFRQLMRMDIAFFDHKNNTPGALTSILAKEAKMIEGLSGATLGQIQQSLVTLIGGIVTGIPFNWRIGLVATSVVPVMLVCGFVRVWVLTQLSDRAREVYERSGSMASEYTSAVRTVQSLTRELDVVVKYTKTVDSQIFSSRIAIARSALYYALSEGMTPWVVALVFWWGSTVMRRGEASVAGYMTVFMAIITGSQAAGQIFSYAPNMNSAKDAARNIYRILTATPSIDVWSEEGYVAPEESVRGDIEFRHVNFRYPTRPQVPVLQDLNLTVKKGQYIALVGASGCGKSTTIGLVERFYDPLAGQVLFDGKDLREYNLNALRSHIALVQQEPMLYSGTLRENILMGWSGPESEVTQEMIEDAARKANIHEFIMSLPDGYETLSGSRGSLLSGGQKQRIAIARALIRNPKVLLLDEATSALDSESEKVVQAALDAAAKGRTTIAVAHRLSTIQKADVIYVFSGGRIVEQGDHQSLLELNGWYAELVNLQGLGEI